European Patent Specification EP 3 838 914 B1, published July 29, 2026. Title: A NOVEL PAENIBACILLUS STRAIN, ANTIFUNGAL COMPOUNDS, AND METHODS FOR THEIR USE. Applicant: Bayer CropScience LP. The sequence listing filed with the application follows.

SEQUENCE LISTING (20 sequences)

SEQ ID NO: 1 - protein, 550 aa, Paenibacillus peoriae
NALVYDPVTIEQIKGHLVHLMEQIVENPAISVDALELVTPQEREQILNVWGNTKGIYEHCNTFHGLLEEQAGRTPDATAIWFEDESLTYAELNAKANGLARRLRTQGIKTGDLVGLIAERSLEMIVGIYGIMKAGGAYVPIDPEYPKERISYMLEDSGAKLILTQAHFLEHLGWTENVLLLDESSTYDADTSNLEDTAGPDDLAYVIYTSGTTGQPKGVLVEHRGLPNLSDVYGAHFEVTPQDRIVQFASLSFDASVSEILTALSHGGVLCIPSTEDILDHALFEQFMNDKGVTVATLPPAYAIHLDPERLPTLRCLLTAGSAASVELIEEWRKHVRYSNGYGPTEDSVCTTIWSVPDSEEATDIVSIGRPIANHSVYILDDHFRLQPVGVAGELCISSIGLARGYHNQPELMDEKFVDNPFAPGERMYRTGDLVRWLPNGTIEYLGRIDHQVKIRGYRIELGEVEAQMLRVPSVQEVVAMAAEGEDGYKDLVAYFVAAQKLEVSELRAVLSEMLPGYMIPSRFIQLEDMPLTSNGKIDRKALQGERGWA

SEQ ID NO: 2 - protein, 550 aa, Paenibacillus polymyxa
NALVYDQVTIGQIKGHLVHLMEQIVENPAISVDALELVTPQEREQILNVWGNMKGIYEHCNTFHGLLEEQAGRTPDATAIWFEDESLTYAELNAKANGLARRLRTQGIKTGDLVGLIAERSLEMIVGIYGIMKAGGAYVPIDPEYPKERISYMLEDSGAKLILTQAHLLEHLGWTENVLLLDESSTYDADTSNLEDTAGPDDLAYVIYTSGTTGQPKGVLVEHRGLPNLSNVYGAHFEVTPQDRIVQFASLSFDASVSEILTALSHGGVLCIPSTEDILDHALFEQFMNDKGITVATLPPAYAIHLDPERLPTLRCLLTAGSAASVELIEEWRKHVRYSNGYGPTEDSVCTTIWSVPDSEEATDIVSIGRPIANHSVYILDDHFRLQPVGVAGELCISSIGLARGYHNRPELMDEKFVDNPFAPGERMYRTGDLVRWLPNGTIEYLGRIDHQVKIRGYRIELGEVEAQMLRVPSVQEVVAMAVEGDDGYKDLVAYFVAAQKLEVSELRAVLSEILPGYMIPSRFIQLEDMPLTSNGKIDRKALQGERGWA

SEQ ID NO: 3 - protein, 550 aa, Paenibacillus polymyxa
NALVYDPVTIEQIKGHLVHLMEQIVENPAISVDALELVTPQEREQILNVWGNTKGIYEHCNTFHGLLEEQAGRTPDATAIWFEDESLTYAELNAKANGLARRLRTQGIKTGDLVGLIAERSLEMIVGIYGIMKAGGAYVPIDPEYPKERISYMLEDSGAKLILTQAHLLEHLGWTENVLLLDESSTYDADTSNLEDTAGPDDLAYVIYTSGTTGQPKGVLVEHRGLPNLSDVYGTHFEVTPQDRIVQFASLSFDASVSEILTALSHGGVLCIPSTQDILDHALFEQFMNDKGITVATLPPAYAIHLDPERLPTLRCLLTAGSAASVELIEEWRKHVRYSNGYGPTEDSVCTTIWSVPDSEEATDIVSIGRPIANHSVYILDDHFRLQPVGVAGELCISSIGLARGYHNRPELMDEKFVDNPFAPGERMYRTGDLVRWLPNGTIEYLGRIDHQVKIRGYRIELGEVEAQMLRVPSVQEVVAMAVEGDDGYKDLVAYFVAAQKLEVSELRAVLSEMLPGYMIPSRFIQLEDMPLTSNGKIDRKALKGERGWA

SEQ ID NO: 4 - protein, 550 aa, Paenibacillus polymyxa
NALVYDPVTIGQIKGHLVHLMEQIVENPAISVDALELITPQEREQILNVWGNTKAIYEHYNTFHGLLEEQAGRTPDAAAIWFEDESLTYAELNAKANGLARRLRTQGIKTGDLVGLIAERSLEMIVGIYGIMKAGGAYVPIDPEYPQERISYMLEDSGAKLILTQAHLLEHLGWTENVLLLDESSTYDADTSNLEDTAGPDDLAYVIYTSGTTGQPKGVLVEHRGLPNLSDVYGAHFEVTPQDRIVQFASLSFDASVSEILTALSHGGVLCIPSAQDILDHALFEQFMNDKGITVATLPPAYAIHLDPERLPTLRCLLTAGSTASIELIEEWRKHVRYSNGYGPTEDSVCTTIWSVPDSEEATNIVSIGRPIANHSVYILDDHFRLQPVGVAGELCISSIGLARGYHNRPELMDEKFVDNPFAPGERMYRTGDLVRWLPNGNIEYLGRIDHQVKIRGYRIELGEVEAQMLRVPSVQEVVAMAVEGDDGYKDLVAYFVAAQKLEVSELRAVLSEMLPGYMIPSRFIQLEDMLLTSNGKIDRKALQGERGWA

SEQ ID NO: 5 - protein, 550 aa, Paenibacillus polymyxa
NALVYDQVTIEQIKEHLVHLMEQIIENPATSVDALELVTPQEREQILNVWGNTNVCYEHNSTFHGLLEEQAGRTPDATALLFGDEMLTYAELNAKANGLARRLRTQGIKTGDLVGLIAERSLEMIVGIYGIMKAGGAYVPIDPEYPKERISYMLEDSGAKLILTQAHLLEHLGWTESVLLLDESSTYDADTSKLEDTAGPDDLAYVIYTSGTTGQPKGVLVEHRGLPNLSDVYGAHFEVTPQDRIVQFASLSFDASVSEILTALSHGGVLCIPSTQDILDHVLFEQFMNDKGITVATLPPAYAIHLDPERLPTLRCLLTAGSAASVELIEEWRKHVRYSNGYGPTEDSVCTTIWSVPDSEGATDIVSIGRPIANHSVYILDDHFRLQPVGVAGELCISGIGLARGYHNQPELMDEKFVDNPFAPGERMYRTGDLVRWLPNGTIEYLGRIDHQVKIRGYRIELGEVEAQILRVPSVQEVVAMAVEGDDGYKDLVAYFVAAQKLEVSELRAVLSEMLPGYMIPSRFIQLDDMPLTSNGKVDRKALQGERGWA

SEQ ID NO: 6 - protein, 550 aa, Paenibacillus polymyxa
NALVYDPATIEQIKGHLFHLMEQIVENPAISVDALELVTPQEREQILSVWGETEASSKHRTTFHGLLEEQAARTPDATAILFENEMLTYAELNAKANGLARRLRAEGIKTGDLVGLLVERSTDMIVGMYGIMKAGGAYVPIDPEYPKERINYMLEDSGTKMILTQAHLLEHIGWMGNVLLLEEPSTYDADESNLKDTADSDDLAYVIYTSGTTGQPKGVLVEHRGLRNLSDVYRGLFEVTPQDRIVQFASLSFDASVSEIITALSHGATLCIPSTQDILDHALFEQFMNSKAITIATLPPAYIIHLEPERLPALRCLLTAGSATSVELIEKWRKHVQYFNGYGPTEDSVCTTMWTVPDSEETMERVSIGQPIANHRVYILDDHFRVLPVGVAGELCISGIGLARGYHNQPALMDEKFVDNPFTPGERMYRTGDLVRWLPDGTIEYLGRIDHQVKIRGYRIELGEVEAHMLRVPFVQEVVALAVESEDGYKDLVAYFVAAQKLEVSELRAVLSEMLPGYMIPSRFVQLEDMPLTSNGKIDRKALQGEQGWA

SEQ ID NO: 7 - protein, 550 aa, Paenibacillus polymyxa
NALVYDPSTIEQIKGHLFHLMEQIVENPAISVDALELVTPQEREQILNVWGETEASSKHRTTFHGLLEEQAARTPDATAILFENEMLTYAELNAKANGLARRLRAEGIKTGDLVGLLVERSTDMIVGMYGIMKAGGAYVPMDPEYPKERINYMLEDSGTKMILAQAHLLEHIDWMGNVLLLEEPSTYDADESNLKDTANSDDLAYVIYTSGTTGQPKGVLVEHRGLRNLSDVYRGLFEVTPQDRIVQFASLSFDASVSEIITALSHGATLCIPSTQDILDHALFEQFMNSKAITIATLPPAYIIHLEPERLPALRCLLTAGSATSVELIEKWRKHVQYFNGYGPTEDSVCTTMWTVPDSEETMERVSIGQPIANHRVYILDDHFRVLPVGVAGELCISGIGLARGYHNQPALMDEKFVDNPFTPGERMYRTGDLVRWLPDGTIEYLGRIDHQVKIRGYRIELGEVEAHMLRVPFVQEVVALAVESEDGYKDLVAYFVAAQKLEVSELRAVLSEMLPGYMIPSRFVQLEDMPLTSNGKIDRKALQGEQGWA

SEQ ID NO: 8 - protein, 550 aa, Paenibacillus polymyxa
NALVYDPATIEQIKGHLFHLMEQIVENPAISVDALELVTPQEREQILNVWGDTGASSKHRTTFHGLLEEQAGRTPDATAIVFENEVLTYAELNAKANGLARRLRAEGIKTGDLVGLIVERSTDMIVGMYGIMKAGGAYVPIDPEYPKERINYMLEDSGTKMILAQAHLLEHRGWTGNVLLLDEPSTYDADTSNLKDTADPDDLAYVIYTSGTTGRPKGVLVEHRGLQNLSDVYRGLFEVTPQDRIVQFASLSFDASVSEILTTLSHGATLCIPSTQEILDHALFEQFMNDKGITVATLPPAYAIHLEPERLPTLRCLLTAGSATSVELIEKWRKHVQYFNAYGPTEDSVCTTIWNAQNSEETVGIVSIGQPIANHRVYILDEHFRLLPVGVAGELCISGIGLARGYHNRPELMDEKFVDNPYAPGERMYRTGDLVRWLSNGTIEYLGRIDHQVKIRGYRIELGEVEAHMLRVPSVQEVVVLAVESDDGYKDLVAYFVAAQKLEVSELRADLSEMLPGYMIPSRFIQLEDMPLTSNGKIDRKALQGERGWA

SEQ ID NO: 9 - protein, 550 aa, Paenibacillus polymyxa; identical to SEQ ID NO: 8

SEQ ID NO: 10 - protein, 250 aa, Paenibacillus sp.
NTLVYDSSNIERIRGHLVHLMEQIVKNPGISVDALELVTPQERDHILNIWKDIAVPYEHYAELHAQAQTAPIGQPNVYIVDDHFRLLPVGVAGELCIAGVGFTREHHNHPELTDEKFVDNPFAPGERMYRTGDLARWLPDGTIQYLGRVDHQVKIRGYRVELSEVEAQMLKVQSVQDVVVMAVEGDDGHKDLFAYFVADQTIEISELRAVLSELLPVYMIPSHFVQLENPLLTPSGKIDRKALQGERGWA

SEQ ID NO: 11 - protein, 550 aa, Paenibacillus sp.
NALVYDQVTIEQIKGHLVHLMEQIVENPAISVDALELVTPQERELILDVWGNTKVSYEHCNTFHGLLEEQAGRTPEATAIVFEDEMLTYAELNAKANGLARKLRNQGIQTGDLVGLIADRSSEMIVGIYGIMKAGGAYVPIDPEYPKERISYMLEDSGAKLVLTQARLLEHLGWTENVLLLDEPSTYDADTSNLKDTVGPDNLAYVIYTSGTTGQPKGVLVEHRGLQNLSDVYGTYFEVTPQDRIVQFASLSFDASVSEVLTALSHGAALCIPSTQDILDYALFEQFINDKGITIATLPPAYAIHLEPERLPALRCLLTAGSAASVELIEKWRKHVRYSNGYGPTEDSICTTIWSVPDSEETLETVSIGRPIANHSVYVLDEHLRLQPVGVVGELCISGIGLARGYHNRPALMDEKFVENPFTPGERMYRTGDLVRWLPNGTIEYVGRIDHQVKIRGYRIELGEVEAQMLRVQSVQEVVAMAVEGDDGQKDLVAYFVAARELEVSELQTVLSEMLPGYMIPSRFIQLEDMPLTSNGKINRKALQGERGWA

SEQ ID NO: 12 - DNA, 804 bp, Paenibacillus sp.
ttgcaaaaaattgaggtattgttggctgatgacaaccgggaatttacgaatctgcttgccgaatatatttccgatcaggagcatatggaagttacaggaatcgcctataatggtgaagaagtgctccaacacatcgcagaatcccgcaacgtacctgatgtacttattttagatattatcatgcctcatctggatggtctcggcgtattggagcgcttgagagaaatgaacctgtctccacagccgaaaatcattatgctgactgcattcggtcaagaaaatattacgcaaagagccgtacagctcggggcatcttattatattttgaagccgtttgacatggaagtgcttcccaaccgtgttcgtcaattggtgggaccacaattagtcagcagcagtccggtgacggtttcttccatgcggtctaatgtggtgccaatcggcaaaacgaaaaacctggatgccagtattacggccattatccatgaaatcggtgtgccagctcatattaagggctatcaatatttacgcgaagccattactatcgtgtacaataatatcgaaattttgggtgccatcaccaaaacattatatcccgcaatcgccgaaaaatttaaaacgacggcatcccgcgtggaacgcgccattcgtcatgccatcgaggtagcatggacacgtggcaacatcgacagcatctctcatctgttcggctacaccattaatatctccaaatccaagccgaccaactcagagtttattgcgatggtagctgacaagcttcggattgagaataaggtgtcctga

SEQ ID NO: 13 - DNA, 804 bp, Paenibacillus sp.
ttgcaaaaaattgaggtattgttggctgatgacaaccgggaatttacgaatctgcttgccgaatatatttccgatcaggagcatatggaagttacaggaatcgcctataatggtgaagaagtgctccaacacatcgcagaatcccgcaacgtacctgatgtacttattttagatattatcatgcctcatctggatggtctcggcgtattggagcgcttgagagaaatgaacctgtctccacagccgaaaatcattatgctgactgcattcggtcaagaaaatattacgcaaagagccgtacagctcggggcatcttattatattttgaagccgtttgacatggaagtgcttcccaaccgtgttcgtcaattggtgggaccacaattagtcagcagcagtccggtgacggtttcttccatgcggtctaatgtggtgccaatcggcaaaacgaaaaacctggatgccagtattacggccattatccatgaaatcggtgtgccagctcatattaagggctatcaatatttacgcgaagccattactatcgtgtacaataatatcgaaattttgggtgccatcaccaaaacattatatcccgcaatcgccgaaaaatttaaaacgacggcatcccgcgtggaacgcgccattcgtcatgccatcgaggtagcatggacacgtggcaacatcgacagcatctctcatctgttcggctacaccattaatatctccaaatccaagccgaccaactcagagtttattgcgatggtagttgacaagcttcggattgagaataaggtgtcctga

SEQ ID NO: 14 - protein, 267 aa, Paenibaciluss terrae
MQKIEVLLADDNREFTNLLAEYISDQEDMEVTGIAYNGEEVLQHIAESRNVPDVLILDIIMPHLDGLGVLERLREMNLSPQPKIIMLTAFGQENITQRAVQLGASYYILKPFDMEVLANRVRQLVGPQLVSSSPLTVSSMRSNVVPMGKTKNLDASITAIIHEIGVPAHIKGYQYLREAITMVYNNIEILGAITKTLYPAIAEKFKTTASRVERAIRHAIEVAWTRGNIDSISHLFGYTINISKSKPTNSEFIAMVADKLRIENKVS

SEQ ID NO: 15 - protein, 267 aa, Paenibacillus sp.
LQKIEVLLADDNREFTNLLAEYISDQEDMEVTGIAYNGEEVLQHIAESRNVPDVLILDIIMPHLDGLGVLERLREMNLSPQPKIIMLTAFGQENITQRAVQLGASYYILKPFDMEVLANRVRQLVGPQLVSSSPVTVSSMRSNVVPMGKTKNLDASITAIIHEIGVPAHIKGYQYLREAITMVYNNIEILGAITKTLYPAIAEKFKTTASRVERAIRHAIEVAWTRGNIDSISHLFGYTINISKSKPTNSEFIAMVADKLRIENKVS

SEQ ID NO: 16 - protein, 267 aa, Paenibacillus sp.
LQKIEVLLADDNREFTNLLAEYISDQEDMEVTGIAYNGEEVLQHIAESRNVPDVLILDIIMPHLDGLGVLERLREMNLSPQPKIIMLTAFGQENITQRAVQLGASYYILKPFDMEVLANRVRQLVGPQLVSSSPVTVSSMRSNVVPMGKTKNLDASITAIIHEIGVPAHIKGYQYLREAITMVYNNIEILGAITKTLYPAIAEKFKTTASRVERAIRHAIEVAWTRGNIDSISHLFGYTINISKSKPTNSEFIAMVVDKLRIENKVS

SEQ ID NO: 17 - protein, 267 aa, Paenibacillus polymyxa
MQKIEVLLADDNREFTNLLAEYISDQEDMEVTGIAYNGEEVLQRIAESRNVPDVLILDIIMPHLDGLGVLERLREMNLTPQPKIIMLTAFGQENITQRAVQLGASYYILKPFDMEVLANRVRQLVGPQLVSSSPVTVSSMRSNVVPMGKTKNLDASITAIIHEIGVPAHIKGYQYLREAITMVYNNIEILGAITKTLYPAIAEKFKTTASRVERAIRHAIEVAWTRGNIDSISHLFGYTINISKSKPTNSEFIAMVVDKLRIENKVS

SEQ ID NO: 18 - protein, 267 aa, Bacillus subtilis
MEKIKVCVADDNRELVSLLSEYIEGQEDMEVIGVAYNGQECLSLFKEKDPDVLVLDIIMPHLDGLAVLERLRESDLKKQPNVIMLTAFGQEDVTKKAVDLGASYFILKPFDMENLVGHIRQVSGNASSVTHRAPSSQSSIIRSSQPEPKKKNLDASITSIIHEIGVPAHIKGYLYLREAISMVYNDIELLGSITKVLYPDIAKKFNTTASRVERAIRHAIEVAWSRGNIDSISSLFGYTVSMTKAKPTNSEFIAMVADKLRLEHKAS

SEQ ID NO: 19 - protein, 264 aa, Bacillus cereus
MEKIKVCLVDDNKELVSMLESYVAAQDDMEVIGTAYNGQECLNLLKDKQPDVLVLDIIMPHLDGLAVLEKMRHIERLRQPSVIMLTAFGQEDVTKKAVDLGASYFILKPFDMENLTSHIRQVSGKANATIKRPLPSFRSATTVDGKPKNLDASITSIIHEIGVPAHIKGYMYLREAISMVYNDIELLGSITKVLYPDIAKKYNTTASRVERAIRHAIEVAWSRGNIDSISSLFGYTVSMSKAKPTNSEFIAMVADKLRLEHKAS

SEQ ID NO: 20 - protein, 273 aa, Clostridium pasteurianum
MEYSKISVLIADDNKEFCNILNDYLLNQSDIVVVGIAKDGIEALKLIEEKKPDLVILDIIMPNMDGLVVLEKLANINIDPVPNVIVLSAVGQDKITQRAITLGADYYVVKPFDMDVFTKRIRQMFNNTILDSETKKTMPISEKAADVKISQSVPLDLEDESIIHEIGVPAHIKGYMYLREAINMVVDNIELLSAVTKELYPSIAKKYNTTASRVERAIRHAIEVAWSRGQVDTINKLFGYTIHNGKGKPTNSEFIAMIADKLRLKNKVKNVAQ